European Patent Specification EP 3 765 504 B1, published July 31, 2024. Title: ANTI-CD25 ANTIBODY AGENTS. Applicant: Tusk Therapeutics Ltd Cancer Research Technology Ltd. The sequence listing filed with the application follows.

SEQUENCE LISTING (21 sequences)

SEQ ID NO: 1 - protein, 272 aa, Homo sapiens
MDSYLLMWGLLTFIMVPGCQAELCDDDPPEIPHATFKAMAYKEGTMLNCECKRGFRRIKSGSLYMLCTGNSSHSSWDNQCQCTSSATRNTTKQVTPQPEEQKERKTTEMQSPMQPVDQASLPGHCREPPPWENEATERIYHFVVGQMVYYQCVQGYRALHRGPAESVCKMTHGKTRWTQPQLICTGEMETSQFPGEEKPQASPEGRPESETSCLVTTTDFQIQTEMAATMETSIFTTEYQVAVAGCVFLLISVLLLSGLTWQRRQRKSRRTI

SEQ ID NO: 2 - protein, 9 aa, Homo sapiens
FTFSSYGMH

SEQ ID NO: 3 - protein, 17 aa, Homo sapiens [sequence omitted]

SEQ ID NO: 4 - protein, 14 aa, Homo sapiens
ARDLGYGDYAAHDY

SEQ ID NO: 5 - protein, 121 aa, Homo sapiens
QVQLVESGGGVVQPGRSLRLSCAASGFTFSSYGMHWVRQAPGKGLEWVAVIWYDGSNKGYADSVKGRFTISRDNSKNTLYLQMNSLRAEDTAVYYCARDLGYGDYAAHDYWGQGTLVTVSS

SEQ ID NO: 6 - protein, 11 aa, Homo sapiens
RASQSISSWLA

SEQ ID NO: 7 - protein, 7 aa, Homo sapiens
KASSLES

SEQ ID NO: 8 - protein, 9 aa, Homo sapiens
QQHNTHPYT

SEQ ID NO: 9 - protein, 107 aa, Homo sapiens
DIQMTQSPSTLSASVGDRVTITCRASQSISSWLAWYQQKPGKAPKLLIYKASSLESGVPSRFSGSGSGTEFTLTISSLQPDDFATYYCQQHNTHPYTFGGGTKVEIK

SEQ ID NO: 10 - protein, 9 aa, Homo sapiens
FTFASYGMH

SEQ ID NO: 11 - protein, 9 aa, Homo sapiens
FTFPSYGMH

SEQ ID NO: 12 - protein, 17 aa, Homo sapiens
VIWYDASTKYYADSVKG

SEQ ID NO: 13 - protein, 17 aa, Homo sapiens
VIWYDAINKYYADSVKG

SEQ ID NO: 14 - protein, 17 aa, Homo sapiens
VIWYDAVNKYYADSVKG

SEQ ID NO: 15 - protein, 17 aa, Homo sapiens
VIWYDALNKYYADSVKG

SEQ ID NO: 16 - protein, 121 aa, Homo sapiens
EVQLVESGGGLVKPGGSLRLSCAASGFTFASYGMHWVRQAPGKGLEWVAVIWYDASTKYYADSVKGRFTISRDNSKNTLYLQMNSLRAEDTAVYYCARDLGYGDYAAHDYWGQGTLVTVSS

SEQ ID NO: 17 - protein, 121 aa, Homo sapiens
QVQLVESGGGLVQPGGSLRLSCAASGFTFPSYGMHWVRQAPGKGLEWVAVIWYDAINKYYADSVKGRFTISRDNSKNTLYLQMNSLRAEDTAVYYCARDLGYGDYAAHDYWGQGTLVTVSS

SEQ ID NO: 18 - protein, 121 aa, Homo sapiens
QVQLVESGGGVVQPGRSLRLSCAASGFTFPSYGMHWVRQAPGKGLEWVAVIWYDAVNKYYADSVKGRFTISRDNSKNTLYLQMNSLRAEDTAVYYCARDLGYGDYAAHDYWGQGTLVTVSS

SEQ ID NO: 19 - protein, 121 aa, Homo sapiens
QVQLVESGGGVVQPGRSLRLSCAASGFTFPSYGMHWVRQAPGKGLEWVAVIWYDASTKYYADSVKGRFTISRDNSKNTLYLQMNSLRAEDTAVYYCARDLGYGDYAAHDYWGQGTLVTVSS

SEQ ID NO: 20 - protein, 121 aa, Homo sapiens
EVQLLESGGGLVQPGGSLRLSCAASGFTFPSYGMHWVRQAPGKGLEWVAVIWYDALNKYYADSVKGRFTISRDNSKNTLYLQMNSLRAEDTAVYYCARDLGYGDYAAHDYWGQGTLVTVSS

SEQ ID NO: 21 - protein, 15 aa, Homo sapiens
KEGTMLNCECKRGFR